European Patent Specification EP 4 034 562 B1, published October 29, 2025. Title: ANTIGEN BINDING PROTEINS. Applicant: GlaxoSmithKline Intellectual Property Development Limited. The sequence listing filed with the application follows.

SEQUENCE LISTING (180 sequences)

SEQ ID NO: 1 - protein, 106 aa, Artificial
  42Y073-86F08-1 variable light chain amino acid sequence
DIQLTQSPSSLSASVGDRVTITCRASQSISSYLNWYQQKPGKAPKLLIYAASSLQSGVPSRFSGSGSGTDFTLTISSLQPEDFATYYCQQVLHTITFGGGTKVEIK

SEQ ID NO: 2 - protein, 122 aa, Artificial
  42Y073-86F08-1 variable heavy chain amino acid sequence
QVQLVQSGAEVKKPGSSVKVSCKASGGTFSSYAISWVRQAPGQGLEWMGGIIPIFGTASYAQKFQGRVTITADESTSTAYMELSSLRSEDTAVYYCARGAGYYGDKDPMDVWGQGTTVTVSS

SEQ ID NO: 3 - DNA, 318 bp, Artificial
  42Y073-86F08-1 variable light chain nucleic acid sequence
gacatccagctgacccagagccctagcagcctgagcgccagcgtgggagacagggtgaccatcacctgcagggccagccagtccatcagcagctacctgaactggtaccagcagaagcccggcaaggcccccaagctgctgatctacgccgcaagctcactgcagagcggcgtgccctctaggtttagcggcagcggcagcggcaccgacttcaccctgaccatcagcagcctccagcccgaggacttcgccacctactactgccagcaggtgctgcacaccatcactttcggcggcggcaccaaggtggagattaag

SEQ ID NO: 4 - DNA, 366 bp, Artificial
  42Y073-86F08-1 variable heavy chain nucleic acid sequence
caggtgcagctggtgcagagcggcgccgaggtgaaaaagcccggcagcagcgtgaaggtgagctgcaaggcctccggcgggaccttcagcagctacgccatcagctgggtgaggcaggctcccggacagggcctggagtggatgggcggcatcatccccattttcggcaccgccagctacgcccagaagttccagggaagggtcaccatcaccgccgacgagagcaccagcaccgcctacatggaactcagcagcctgaggagcgaggacaccgccgtgtactattgcgccaggggcgccggctactacggcgacaaggaccccatggacgtgtggggccagggcaccaccgtgactgtgagcagc

SEQ ID NO: 5 - protein, 107 aa, Artificial
  42Y073-86F04-3 variable light chain amino acid sequence
DIQMTQSPSSLSASVGDRVTITCRASQSISSYLNWYQQKPGKAPKLLIYAASSLQSGVPSRFSGSGSGTDFTLTISSLQPEDFATYYCQQPYFSPPTFGGGTKVEIK

SEQ ID NO: 6 - protein, 118 aa, Artificial
  42Y073-86F04-3 variable heavy chain amino acid sequence
QVQLVQSGAEVKKPGSSVKVSCKASGGTFSYNAISWVRQAPGQGLEWMGGIIPIMGTARYAQKFQGRVTITADESTSTAYMELSSLRSEDTAVYYCARLLGESGMDVWGQGTTVTVSS

SEQ ID NO: 7 - DNA, 321 bp, Artificial
  42Y073-86F04-3 variable light chain nucleic acid sequence
gacatccagatgacccagagccctagcagcctgagcgccagcgtgggagacagggtgaccatcacctgcagggccagccagtccatcagcagctacctgaactggtaccagcagaagcccggcaaggcccccaagctgctgatctacgccgcaagctcactgcagagcggcgtgccctctaggtttagcggcagcggcagcggcaccgacttcaccctgaccatcagcagcctccagcccgaggacttcgccacctactactgccagcagccctacttcagcccccccactttcggcggcggcaccaaggtggagattaag

SEQ ID NO: 8 - DNA, 354 bp, Artificial
  42Y073-86F04-3 variable heavy chain nucleic acid sequence
caggtgcagctggtgcagagcggcgccgaggtgaaaaagcccggcagcagcgtgaaggtgagctgcaaggcctccggcgggaccttcagctacaacgccatcagctgggtgaggcaggctcccggacagggcctggagtggatgggcggcatcatccccattatgggcaccgccaggtacgcccagaagttccagggaagggtcaccatcaccgccgacgagagcaccagcaccgcctacatggaactcagcagcctgaggagcgaggacaccgccgtgtactattgcgccaggctgctgggcgagagcggcatggacgtgtggggccagggcaccaccgtgactgtgagcagc

SEQ ID NO: 9 - protein, 107 aa, Artificial; identical to SEQ ID NO: 5
  42Y073-86F04-4 variable light chain amino acid sequence

SEQ ID NO: 10 - protein, 118 aa, Artificial
  42Y073-86F04-4 variable heavy chain amino acid sequence
QVQLVQSGAEVKKPGSSVKVSCKASGGTFESEAISWVRQAPGQGLEWMGGIIPIFGRARYAQKFQGRVTITADESTSTAYMELSSLRSEDTAVYYCARLLGESGMDVWGQGTTVTVSS

SEQ ID NO: 11 - DNA, 321 bp, Artificial; identical to SEQ ID NO: 7
  42Y073-86F04-4 variable light chain nucleic acid sequence

SEQ ID NO: 12 - DNA, 354 bp, Artificial
  42Y073-86F04-4 variable heavy chain nucleic acid sequence
caggtgcagctggtgcagagcggcgccgaggtgaaaaagcccggcagcagcgtgaaggtgagctgcaaggcctccggcgggaccttcgagagcgaggccatcagctgggtgaggcaggctcccggacagggcctggagtggatgggcggcatcatccccattttcggcagggccaggtacgcccagaagttccagggaagggtcaccatcaccgccgacgagagcaccagcaccgcctacatggaactcagcagcctgaggagcgaggacaccgccgtgtactattgcgccaggctgctgggcgagagcggcatggacgtgtggggccagggcaccaccgtgactgtgagcagc

SEQ ID NO: 13 - protein, 107 aa, Artificial; identical to SEQ ID NO: 5
  42Y073-86F04-5 variable light chain amino acid sequence

SEQ ID NO: 14 - protein, 118 aa, Artificial
  42Y073-86F04-5 variable heavy chain amino acid sequence
QVQLVQSGAEVKKPGSSVKVSCKASGGTFSSHAISWVRQAPGQGLEWMGGIIPIFGRGKYAQKFQGRVTITADESTSTAYMELSSLRSEDTAVYYCARLLGESGMDVWGQGTTVTVSS

SEQ ID NO: 15 - DNA, 321 bp, Artificial; identical to SEQ ID NO: 7
  42Y073-86F04-5 variable light chain nucleic acid sequence

SEQ ID NO: 16 - DNA, 354 bp, Artificial
  42Y073-86F04-5 variable heavy chain nucleic acid sequence
caggtgcagctggtgcagagcggcgccgaggtgaaaaagcccggcagcagcgtgaaggtgagctgcaaggcctccggcgggaccttcagcagccacgccatcagctgggtgaggcaggctcccggacagggcctggagtggatgggcggcatcatccccattttcggcaggggcaagtacgcccagaagttccagggaagggtcaccatcaccgccgacgagagcaccagcaccgcctacatggaactcagcagcctgaggagcgaggacaccgccgtgtactattgcgccaggctgctgggcgagagcggcatggacgtgtggggccagggcaccaccgtgactgtgagcagc

SEQ ID NO: 17 - protein, 107 aa, Artificial; identical to SEQ ID NO: 5
  42Y073-86F04-6 variable light chain amino acid sequence

SEQ ID NO: 18 - protein, 118 aa, Artificial
  42Y073-86F04-6 variable heavy chain amino acid sequence
QVQLVQSGAEVKKPGSSVKVSCKASGGTFSGHAISWVRQAPGQGLEWMGGIIPIFGRARYAQKFQGRVTITADESTSTAYMELSSLRSEDTAVYYCARLLGESGMDVWGQGTTVTVSS

SEQ ID NO: 19 - DNA, 321 bp, Artificial; identical to SEQ ID NO: 7
  42Y073-86F04-6 variable light chain nucleic acid sequence

SEQ ID NO: 20 - DNA, 354 bp, Artificial
  42Y073-86F04-6 variable heavy chain nucleic acid sequence
caggtgcagctggtgcagagcggcgccgaggtgaaaaagcccggcagcagcgtgaaggtgagctgcaaggcctccggcgggaccttcagcggccacgccatcagctgggtgaggcaggctcccggacagggcctggagtggatgggcggcatcatccccattttcggcagggccaggtacgcccagaagttccagggaagggtcaccatcaccgccgacgagagcaccagcaccgcctacatggaactcagcagcctgaggagcgaggacaccgccgtgtactattgcgccaggctgctgggcgagagcggcatggacgtgtggggccagggcaccaccgtgactgtgagcagc

SEQ ID NO: 21 - protein, 107 aa, Artificial; identical to SEQ ID NO: 5
  42Y073-86F04-18 variable light chain amino acid sequence

SEQ ID NO: 22 - protein, 118 aa, Artificial
  42Y073-86F04-18 variable heavy chain amino acid sequence
QVQLVQSGAEVKKPGSSVKVSCKASGGTFSSRAISWVRQAPGQGLEWMGGIIPIMGTARYAQKFQGRVTITADESTSTAYMELSSLRSEDTAVYYCARLLGESGMDVWGQGTTVTVSS

SEQ ID NO: 23 - DNA, 321 bp, Artificial; identical to SEQ ID NO: 7
  42Y073-86F04-18 variable light chain nucleic acid sequence

SEQ ID NO: 24 - DNA, 354 bp, Artificial
  42Y073-86F04-18 variable heavy chain nucleic acid sequence
caggtgcagctggtgcagagcggcgccgaggtgaaaaagcccggcagcagcgtgaaggtgagctgcaaggcctccggcgggaccttcagcagcagggccatcagctgggtgaggcaggctcccggacagggcctggagtggatgggcggcatcatccccattatgggcaccgccaggtacgcccagaagttccagggaagggtcaccatcaccgccgacgagagcaccagcaccgcctacatggaactcagcagcctgaggagcgaggacaccgccgtgtactattgcgccaggctgctgggcgagagcggcatggacgtgtggggccagggcaccaccgtgactgtgagcagc

SEQ ID NO: 25 - protein, 107 aa, Artificial; identical to SEQ ID NO: 5
  42Y073-86F04-33 variable light chain amino acid sequence

SEQ ID NO: 26 - protein, 118 aa, Artificial
  42Y073-86F04-33 variable heavy chain amino acid sequence
QVQLVQSGAEVKKPGSSVKVSCKASGGTFSSYAISWVRQAPGQGLEWMGGILPIFGRANYAQKFQGRVTITADESTSTAYMELSSLRSEDTAVYYCARLLGESGMDVWGQGTTVTVSS

SEQ ID NO: 27 - DNA, 321 bp, Artificial; identical to SEQ ID NO: 7
  42Y073-86F04-33 variable light chain nucleic acid sequence

SEQ ID NO: 28 - DNA, 354 bp, Artificial
  42Y073-86F04-33 variable heavy chain nucleic acid sequence
caggtgcagctggtgcagagcggcgccgaggtgaaaaagcccggcagcagcgtgaaggtgagctgcaaggcctccggcgggaccttcagcagctacgccatcagctgggtgaggcaggctcccggacagggcctggagtggatgggcggcatcctgcccattttcggcagggccaactacgcccagaagttccagggaagggtcaccatcaccgccgacgagagcaccagcaccgcctacatggaactcagcagcctgaggagcgaggacaccgccgtgtactattgcgccaggctgctgggcgagagcggcatggacgtgtggggccagggcaccaccgtgactgtgagcagc

SEQ ID NO: 29 - protein, 107 aa, Artificial; identical to SEQ ID NO: 5
  42Y073-86F04-88 variable light chain amino acid sequence

SEQ ID NO: 30 - protein, 118 aa, Artificial
  42Y073-86F04-88 variable heavy chain amino acid sequence
QVQLVQSGAEVKKPGSSVKVSCKASGGTFSSSAISWVRQAPGQGLEWMGGIIPIFGRANYAQKFQGRVTITADESTSTAYMELSSLRSEDTAVYYCARLLGESGMDVWGQGTTVTVSS

SEQ ID NO: 31 - DNA, 321 bp, Artificial; identical to SEQ ID NO: 7
  42Y073-86F04-88 variable light chain nucleic acid sequence

SEQ ID NO: 32 - DNA, 354 bp, Artificial
  42Y073-86F04-88 variable heavy chain nucleic acid sequence
caggtgcagctggtgcagagcggcgccgaggtgaaaaagcccggcagcagcgtgaaggtgagctgcaaggcctccggcgggaccttcagcagcagcgccatcagctgggtgaggcaggctcccggacagggcctggagtggatgggcggcatcatccccattttcggcagggccaactacgcccagaagttccagggaagggtcaccatcaccgccgacgagagcaccagcaccgcctacatggaactcagcagcctgaggagcgaggacaccgccgtgtactattgcgccaggctgctgggcgagagcggcatggacgtgtggggccagggcaccaccgtgactgtgagcagc

SEQ ID NO: 33 - protein, 106 aa, Artificial; identical to SEQ ID NO: 1
  42Y073-86F08-3 variable light chain amino acid sequence

SEQ ID NO: 34 - protein, 122 aa, Artificial
  42Y073-86F08-3 variable heavy chain amino acid sequence
QVQLVQSGAEVKKPGSSVKVSCKASGGTFVNYAISWVRQAPGQGLEWMGGIIPALGTANYAQKFQGRVTITADESTSTAYMELSSLRSEDTAVYYCARGAGYYGDKDPMDVWGQGTTVTVSS

SEQ ID NO: 35 - DNA, 318 bp, Artificial; identical to SEQ ID NO: 3
  42Y073-86F08-3 variable light chain nucleic acid sequence

SEQ ID NO: 36 - DNA, 366 bp, Artificial
  42Y073-86F08-3 variable heavy chain nucleic acid sequence
caggtgcagctggtgcagagcggcgccgaggtgaaaaagcccggcagcagcgtgaaggtgagctgcaaggcctccggcgggaccttcgtgaactacgccatcagctgggtgaggcaggctcccggacagggcctggagtggatgggcggcatcatccccgccctgggcaccgccaactacgcccagaagttccagggaagggtcaccatcaccgccgacgagagcaccagcaccgcctacatggaactcagcagcctgaggagcgaggacaccgccgtgtactattgcgccaggggcgccggctactacggcgacaaggaccccatggacgtgtggggccagggcaccaccgtgactgtgagcagc

SEQ ID NO: 37 - protein, 106 aa, Artificial; identical to SEQ ID NO: 1
  42Y073-86F08-4 variable light chain amino acid sequence

SEQ ID NO: 38 - protein, 122 aa, Artificial
  42Y073-86F08-4 variable heavy chain amino acid sequence
QVQLVQSGAEVKKPGSSVKVSCKASGGTFSEYAIHWVRQAPGQGLEWMGNIIPIFGTAGYAQKFQGRVTITADESTSTAYMELSSLRSEDTAVYYCARGAGYYGDKDPMDVWGQGTTVTVSS

SEQ ID NO: 39 - DNA, 318 bp, Artificial; identical to SEQ ID NO: 3
  42Y073-86F08-4 variable light chain nucleic acid sequence

SEQ ID NO: 40 - DNA, 366 bp, Artificial
  42Y073-86F08-4 variable heavy chain nucleic acid sequence
caggtgcagctggtgcagagcggcgccgaggtgaaaaagcccggcagcagcgtgaaggtgagctgcaaggcctccggcgggaccttcagcgagtacgccatccactgggtgaggcaggctcccggacagggcctggagtggatgggcaacatcatccccattttcggcaccgccggctacgcccagaagttccagggaagggtcaccatcaccgccgacgagagcaccagcaccgcctacatggaactcagcagcctgaggagcgaggacaccgccgtgtactattgcgccaggggcgccggctactacggcgacaaggaccccatggacgtgtggggccagggcaccaccgtgactgtgagcagc

SEQ ID NO: 41 - protein, 106 aa, Artificial; identical to SEQ ID NO: 1
  42Y073-86F08-8 variable light chain amino acid sequence

SEQ ID NO: 42 - protein, 122 aa, Artificial
  42Y073-86F08-8 variable heavy chain amino acid sequence
QVQLVQSGAEVKKPGSSVKVSCKASGGTFWLYAISWVRQAPGQGLEWMGGIIPQLGTANYAQKFQGRVTITADESTSTAYMELSSLRSEDTAVYYCARGAGYYGDKDPMDVWGQGTTVTVSS

SEQ ID NO: 43 - DNA, 318 bp, Artificial; identical to SEQ ID NO: 3
  42Y073-86F08-8 variable light chain nucleic acid sequence

SEQ ID NO: 44 - DNA, 366 bp, Artificial
  42Y073-86F08-8 variable heavy chain nucleic acid sequence
caggtgcagctggtgcagagcggcgccgaggtgaaaaagcccggcagcagcgtgaaggtgagctgcaaggcctccggcgggaccttctggctgtacgccatcagctgggtgaggcaggctcccggacagggcctggagtggatgggcggcatcatcccccagctgggcaccgccaactacgcccagaagttccagggaagggtcaccatcaccgccgacgagagcaccagcaccgcctacatggaactcagcagcctgaggagcgaggacaccgccgtgtactattgcgccaggggcgccggctactacggcgacaaggaccccatggacgtgtggggccagggcaccaccgtgactgtgagcagc

SEQ ID NO: 45 - protein, 106 aa, Artificial; identical to SEQ ID NO: 1
  42Y073-86F08-17 variable light chain amino acid sequence

SEQ ID NO: 46 - protein, 122 aa, Artificial
  42Y073-86F08-17 variable heavy chain amino acid sequence
QVQLVQSGAEVKKPGSSVKVSCKASGGTFREYAISWVRQAPGQGLEWMGGIIPVFGTANYAQKFQGRVTITADESTSTAYMELSSLRSEDTAVYYCARGAGYYGDKDPMDVWGQGTTVTVSS

SEQ ID NO: 47 - DNA, 318 bp, Artificial; identical to SEQ ID NO: 3
  42Y073-86F08-17 variable light chain nucleic acid sequence

SEQ ID NO: 48 - DNA, 366 bp, Artificial
  42Y073-86F08-17 variable heavy chain nucleic acid sequence
caggtgcagctggtgcagagcggcgccgaggtgaaaaagcccggcagcagcgtgaaggtgagctgcaaggcctccggcgggaccttcagggagtacgccatcagctgggtgaggcaggctcccggacagggcctggagtggatgggcggcatcatccccgtgttcggcaccgccaactacgcccagaagttccagggaagggtcaccatcaccgccgacgagagcaccagcaccgcctacatggaactcagcagcctgaggagcgaggacaccgccgtgtactattgcgccaggggcgccggctactacggcgacaaggaccccatggacgtgtggggccagggcaccaccgtgactgtgagcagc

SEQ ID NO: 49 - protein, 106 aa, Artificial; identical to SEQ ID NO: 1
  42Y073-86F08-22 variable light chain amino acid sequence

SEQ ID NO: 50 - protein, 122 aa, Artificial
  42Y073-86F08-22 variable heavy chain amino acid sequence
QVQLVQSGAEVKKPGASVKVSCKASGYTFDSYAMHWVRQAPGQGLEWMGGIIPIFGTAWYAQKFQGRVTITADESTSTAYMELSSLRSEDTAVYYCARGAGYYGDKDPMDVWGQGTTVTVSS

SEQ ID NO: 51 - DNA, 318 bp, Artificial; identical to SEQ ID NO: 3
  42Y073-86F08-22 variable light chain nucleic acid sequence

SEQ ID NO: 52 - DNA, 366 bp, Artificial
  42Y073-86F08-22 variable heavy chain nucleic acid sequence
caggtgcagctggtgcagagcggcgccgaggtgaaaaagcccggcgccagcgtgaaggtgagctgcaaggcctccggctacaccttcgacagctacgccatgcactgggtgaggcaggctcccggacagggcctggagtggatgggcggcatcatccccattttcggcaccgcctggtacgcccagaagttccagggaagggtcaccatcaccgccgacgagagcaccagcaccgcctacatggaactcagcagcctgaggagcgaggacaccgccgtgtactattgcgccaggggcgccggctactacggcgacaaggaccccatggacgtgtggggccagggcaccaccgtgactgtgagcagc

SEQ ID NO: 53 - protein, 106 aa, Artificial; identical to SEQ ID NO: 1
  42Y073-86F08-47 variable light chain amino acid sequence

SEQ ID NO: 54 - protein, 122 aa, Artificial
  42Y073-86F08-47 variable heavy chain amino acid sequence
QVQLVQSGAEVKKPGSSVKVSCKASGGTFSQYAIHWVRQAPGQGLEWMGVIIPIFGKANYAQKFQGRVTITADESTSTAYMELSSLRSEDTAVYYCARGAGYYGDKDPMDVWGQGTTVTVSS

SEQ ID NO: 55 - DNA, 318 bp, Artificial; identical to SEQ ID NO: 3
  42Y073-86F08-47 variable light chain nucleic acid sequence

SEQ ID NO: 56 - DNA, 366 bp, Artificial
  42Y073-86F08-47 variable heavy chain nucleic acid sequence
caggtgcagctggtgcagagcggcgccgaggtgaaaaagcccggcagcagcgtgaaggtgagctgcaaggcctccggcgggaccttcagccagtacgccatccactgggtgaggcaggctcccggacagggcctggagtggatgggcgtgatcatccccattttcggcaaggccaactacgcccagaagttccagggaagggtcaccatcaccgccgacgagagcaccagcaccgcctacatggaactcagcagcctgaggagcgaggacaccgccgtgtactattgcgccaggggcgccggctactacggcgacaaggaccccatggacgtgtggggccagggcaccaccgtgactgtgagcagc

SEQ ID NO: 57 - protein, 107 aa, Artificial
  42Y073-2B04-46 variable light chain amino acid sequence
EIVLTQSPATLSLSPGERATLSCRASQSVSSYLAWYQQKPGQAPRLLIYDASKRATGIPARFSGSGSGTDFTLTISSLEPEDFAVYYCQQLDNWPITFGGGTKVEIK

SEQ ID NO: 58 - protein, 126 aa, Artificial
  42Y073-2B04-46 variable heavy chain amino acid sequence
QVQLQQWGAGLLKPSETLSLTCAVYGGSFRRYYWSWIRQPPGKGLEWIGEIDGWGSTNYNPSLKSRVTISVDTSKNQFSLKLSSVTAADTAVYYCARGGSVDFWSGSDYYYYMDVWGKGATVTVSS

SEQ ID NO: 59 - DNA, 321 bp, Artificial
  42Y073-2B04-46 variable light chain nucleic acid sequence
gagatcgtgctgacccagagccccgcaaccctgtccctgagccccggcgaaagggccactctgagctgcagggccagccagagcgtgagcagctacctcgcctggtaccagcagaagcccggccaggcccctaggctgctgatctacgacgccagcaagagggccaccggcattcccgccaggttcagcggcagcggcagcggcaccgacttcaccctgaccatcagcagcctggagcccgaggacttcgccgtctactactgccagcagctggacaactggcccatcaccttcgggggcggcaccaaggtggagatcaag

SEQ ID NO: 60 - DNA, 377 bp, Artificial
  42Y073-2B04-46 variable heavy chain nucleic acid sequence
caggtgcagctgcagcagtggggcgccggactgctgaagcccagcgagaccctgagcctgacctgcgccgtgtacggcgggtccttcaggaggtactactggagctggatcaggcagccccccggcaaaggcctggagtggatcggcgagatcgacggctggggcagcaccaactacaaccccagcctcaagagcagggtgaccatcagcgtggacaccagcaagaaccagttcagcctgaagctgagcagcgtgaccgccgccgacaccgccgtgtactattgcgccaggggcggcagcgtggacttctggagcggcagcgactactactactacatggacgtgtggggcaagggcgccaccgtcaccgtgagcag

SEQ ID NO: 61 - protein, 107 aa, Artificial
  42Y073-1A01-85 variable light chain amino acid sequence
DIQMTQSPSSLSASVGDRVTITCRASQSISSYLNWYQQKPGKAPKLLIYAASSLQSGVPSRFSGSGSGTDFTLTISSLQPEDFATYYCQQSLYPPRTFGGGTKVEIK

SEQ ID NO: 62 - protein, 123 aa, Artificial
  42Y073-1A01-85 variable heavy chain amino acid sequence
QVQLVQSGAEVKKPGASVKVSCKASGYTFTSYPMHWVRQAPGQGLEWMGIINPSGGFTSYAQKFQGRVTMTRDTSTSTVYMELSSLRSEDTAVYYCARETAYYTTKGNWFDPWGQGTLVTVSA

SEQ ID NO: 63 - DNA, 321 bp, Artificial
  42Y073-1A01-85 variable light chain nucleic acid sequence
gacatccagatgacccagagccctagcagcctgagcgccagcgtgggagacagggtgaccatcacctgcagggccagccagtccatcagcagctacctgaactggtaccagcagaagcccggcaaggcccccaagctgctgatctacgccgcaagctcactgcagagcggcgtgccctctaggtttagcggcagcggcagcggcaccgacttcaccctgaccatcagcagcctccagcccgaggacttcgccacctactactgccagcagagcctgtacccccccaggactttcggcggcggcaccaaggtggagattaag

SEQ ID NO: 64 - DNA, 369 bp, Artificial
  42Y073-1A01-85 variable heavy chain nucleic acid sequence
caggtgcagctggtgcagagcggcgccgaagtgaaaaagcccggcgccagcgtgaaggtcagctgcaaggcctccgggtacaccttcaccagctaccccatgcactgggtgaggcaggcccccggccagggcctcgagtggatgggcatcatcaaccccagcggaggcttcaccagctacgcccagaagttccagggcagggtgaccatgacaagggacaccagcaccagcaccgtgtacatggagctgagcagcctgaggagcgaggacaccgccgtgtattactgcgcaagggagaccgcctactacaccaccaagggcaactggttcgacccctggggccagggcaccctggtgaccgtgagcgcc

SEQ ID NO: 65 - protein, 107 aa, Artificial; identical to SEQ ID NO: 61
  42Y073-1A01-97 variable light chain amino acid sequence

SEQ ID NO: 66 - protein, 123 aa, Artificial
  42Y073-1A01-97 variable heavy chain amino acid sequence
QVQLVQSGAEVKKPGASVKVSCKASGYTFTRAAMHWVRQAPGQGLEWMGIINPAGGYTSYAQKFQGRVTMTRDTSTSTVYMELSSLRSEDTAVYYCARETAYYTTKGNWFDPWGQGTLVTVSS

SEQ ID NO: 67 - DNA, 321 bp, Artificial; identical to SEQ ID NO: 63
  42Y073-1A01-97 variable light chain nucleic acid sequence

SEQ ID NO: 68 - DNA, 369 bp, Artificial
  42Y073-1A01-97 variable heavy chain nucleic acid sequence
caggtgcagctggtgcagagcggcgccgaagtgaaaaagcccggcgccagcgtgaaggtcagctgcaaggcctccgggtacaccttcaccagggccgccatgcactgggtgaggcaggcccccggccagggcctcgagtggatgggcatcatcaaccccgccggaggctacaccagctacgcccagaagttccagggcagggtgaccatgacaagggacaccagcaccagcaccgtgtacatggagctgagcagcctgaggagcgaggacaccgccgtgtattactgcgcaagggagaccgcctactacaccaccaagggcaactggttcgacccctggggccagggcaccctggtgaccgtgagctct

SEQ ID NO: 69 - protein, 107 aa, Artificial; identical to SEQ ID NO: 61
  42Y073-1A01-100 variable light chain amino acid sequence

SEQ ID NO: 70 - protein, 123 aa, Artificial
  42Y073-1A01-100 variable heavy chain amino acid sequence
QVQLVQSGAEVKKPGASVKVSCKASGYTFTTYRMHWVRQAPGQGLEWMGIINPSGGLTQYAQKFQGRVTMTRDTSTSTVYMELSSLRSEDTAVYYCARETAYYTTKGNWFDPWGQGTLVTVSS

SEQ ID NO: 71 - DNA, 321 bp, Artificial; identical to SEQ ID NO: 63
  42Y073-1A01-100 variable light chain nucleic acid sequence

SEQ ID NO: 72 - DNA, 369 bp, Artificial
  42Y073-1A01-100 variable heavy chain nucleic acid sequence
caggtgcagctggtgcagagcggcgccgaagtgaaaaagcccggcgccagcgtgaaggtcagctgcaaggcctccgggtacaccttcaccacctacaggatgcactgggtgaggcaggcccccggccagggcctcgagtggatgggcatcatcaaccccagcggaggcctgacccagtacgcccagaagttccagggcagggtgaccatgacaagggacaccagcaccagcaccgtgtacatggagctgagcagcctgaggagcgaggacaccgccgtgtattactgcgcaagggagaccgcctactacaccaccaagggcaactggttcgacccctggggccagggcaccctggtgaccgtgagctct

SEQ ID NO: 73 - protein, 107 aa, Artificial; identical to SEQ ID NO: 61
  42Y073-1A01-103 variable light chain amino acid sequence

SEQ ID NO: 74 - protein, 123 aa, Artificial
  42Y073-1A01-103 variable heavy chain amino acid sequence
QVQLVQSGAEVKKPGASVKVSCKASGYTFTAYQMHWVRQAPGQGLEWMGIINPAGGWTSYAQKFQGRVTMTRDTSTSTVYMELSSLRSEDTAVYYCARETAYYTTKGNWFDPWGQGTLVTVSS

SEQ ID NO: 75 - DNA, 321 bp, Artificial; identical to SEQ ID NO: 63
  42Y073-1A01-103 variable light chain nucleic acid sequence

SEQ ID NO: 76 - DNA, 369 bp, Artificial
  42Y073-1A01-103 variable heavy chain nucleic acid sequence
caggtgcagctggtgcagagcggcgccgaagtgaaaaagcccggcgccagcgtgaaggtcagctgcaaggcctccgggtacaccttcaccgcctaccagatgcactgggtgaggcaggcccccggccagggcctcgagtggatgggcatcatcaaccccgccggaggctggaccagctacgcccagaagttccagggcagggtgaccatgacaagggacaccagcaccagcaccgtgtacatggagctgagcagcctgaggagcgaggacaccgccgtgtattactgcgcaagggagaccgcctactacaccaccaagggcaactggttcgacccctggggccagggcaccctggtgaccgtgagctct

SEQ ID NO: 77 - protein, 107 aa, Artificial; identical to SEQ ID NO: 61
  42Y073-1A01-126 variable light chain amino acid sequence

SEQ ID NO: 78 - protein, 123 aa, Artificial
  42Y073-1A01-126 variable heavy chain amino acid sequence
QVQLVQSGAEVKKPGASVKVSCKASGYTFTRYNMHWVRQAPGQGLEWMGWINPAGGSTSYAQKFQGRVTMTRDTSTSTVYMELSSLRSEDTAVYYCARETAYYTTKGNWFDPWGQGTLVTVSA

SEQ ID NO: 79 - DNA, 321 bp, Artificial; identical to SEQ ID NO: 63
  42Y073-1A01-126 variable light chain nucleic acid sequence

SEQ ID NO: 80 - DNA, 369 bp, Artificial
  42Y073-1A01-126 variable heavy chain nucleic acid sequence
caggtgcagctggtgcagagcggcgccgaagtgaaaaagcccggcgccagcgtgaaggtcagctgcaaggcctccgggtacaccttcaccaggtacaacatgcactgggtgaggcaggcccccggccagggcctcgagtggatgggctggatcaaccccgccggaggcagcaccagctacgcccagaagttccagggcagggtgaccatgacaagggacaccagcaccagcaccgtgtacatggagctgagcagcctgaggagcgaggacaccgccgtgtattactgcgcaagggagaccgcctactacaccaccaagggcaactggttcgacccctggggccagggcaccctggtgaccgtgagcgcc

SEQ ID NO: 81 - protein, 107 aa, Artificial; identical to SEQ ID NO: 61
  42Y073-1A01-191 variable light chain amino acid sequence

SEQ ID NO: 82 - protein, 123 aa, Artificial
  42Y073-1A01-191 variable heavy chain amino acid sequence
QVQLVQSGAEVKKPGASVKVSCKASGYTFTKYRMHWVRQAPGQGLEWMGIINPQGGSTSYAQKFQGRVTMTRDTSTSTVYMELSSLRSEDTAVYYCARETAYYTTKGNWFDPWGQGTLVTVSA

SEQ ID NO: 83 - DNA, 321 bp, Artificial; identical to SEQ ID NO: 63
  42Y073-1A01-191 variable light chain nucleic acid sequence

SEQ ID NO: 84 - DNA, 369 bp, Artificial
  42Y073-1A01-191 variable heavy chain nucleic acid sequence
caggtgcagctggtgcagagcggcgccgaagtgaaaaagcccggcgccagcgtgaaggtcagctgcaaggcctccgggtacaccttcaccaagtacaggatgcactgggtgaggcaggcccccggccagggcctcgagtggatgggcatcatcaacccccagggaggcagcaccagctacgcccagaagttccagggcagggtgaccatgacaagggacaccagcaccagcaccgtgtacatggagctgagcagcctgaggagcgaggacaccgccgtgtattactgcgcaagggagaccgcctactacaccaccaagggcaactggttcgacccctggggccagggcaccctggtgaccgtgagcgcc

SEQ ID NO: 85 - protein, 106 aa, Artificial; identical to SEQ ID NO: 1
  42Y073-86F08-66 variable light chain amino acid sequence

SEQ ID NO: 86 - protein, 122 aa, Artificial
  42Y073-86F08-66 variable heavy chain amino acid sequence
QVQLVQSGAEVKKPGSSVKVSCKASGGTFVEYAISWVRQAPGQGLEWMGGIIPAFGTAQYAQKFQGRVTITADESTSTAYMELSSLRSEDTAVYYCARGAGYYGDKDPMDVWGQGTTVTVSS

SEQ ID NO: 87 - DNA, 318 bp, Artificial; identical to SEQ ID NO: 3
  42Y073-86F08-66 variable light chain nucleic acid sequence

SEQ ID NO: 88 - DNA, 366 bp, Artificial
  42Y073-86F08-66 variable heavy chain nucleic acid sequence
caggtgcagctggtgcagagcggcgcagaggtgaaaaagcccggcagcagcgtgaaggtgagctgcaaggcctccggcgggaccttcgtggagtacgccatcagctgggtgaggcaggctcccggacagggcctggagtggatgggcggcatcatccccgccttcggcaccgcccagtacgcccagaagttccagggaagggtcaccatcaccgccgacgagagcaccagcaccgcctacatggaactcagcagcctgaggagcgaggacaccgccgtgtactattgcgccaggggagccggctactacggcgacaaggaccccatggacgtgtggggccagggcaccaccgtgactgtgagcagc

SEQ ID NO: 89 - protein, 106 aa, Artificial; identical to SEQ ID NO: 1
  42Y073-86F08-16 variable light chain amino acid sequence

SEQ ID NO: 90 - protein, 122 aa, Artificial
  42Y073-86F08-16 variable heavy chain amino acid sequence
QVQLVQSGAEVKKPGSSVKVSCKASGGTFNEYAISWVRQAPGQGLEWMGGIVPVFGTAKYAQKFQGRVTITADESTSTAYMELSSLRSEDTAVYYCARGAGYYGDKDPMDVWGQGTTVTVSS

SEQ ID NO: 91 - DNA, 318 bp, Artificial; identical to SEQ ID NO: 3
  42Y073-86F08-16 variable light chain nucleic acid sequence

SEQ ID NO: 92 - DNA, 366 bp, Artificial
  42Y073-86F08-16 variable heavy chain nucleic acid sequence
caggtgcagctggtgcagagcggcgccgaggtgaaaaagcccggcagcagcgtgaaggtgagctgcaaggcctccggcgggaccttcaacgagtacgccatcagctgggtgaggcaggctcccggacagggcctggagtggatgggcggcatcgtgcccgtgttcggcaccgccaagtacgcccagaagttccagggaagggtcaccatcaccgccgacgagagcaccagcaccgcctacatggaactcagcagcctgaggagcgaggacaccgccgtgtactattgcgccaggggcgccggctactacggcgacaaggaccccatggacgtgtggggccagggcaccaccgtgactgtgagcagc

SEQ ID NO: 93 - protein, 107 aa, Artificial; identical to SEQ ID NO: 5
  42Y073-86F04-23 variable light chain amino acid sequence

SEQ ID NO: 94 - protein, 118 aa, Artificial
  42Y073-86F04-23 variable heavy chain amino acid sequence
QVQLVQSGAEVKKPGSSVKVSCKASGGTFSGYPISWVRQAPGQGLEWMGGIIPIMGTARYAQKFQGRVTITADESTSTAYMELSSLRSEDTAVYYCARLLGESGMDVWGQGTTVTVSS

SEQ ID NO: 95 - DNA, 321 bp, Artificial; identical to SEQ ID NO: 7
  42Y073-86F04-23 variable light chain nucleic acid sequence

SEQ ID NO: 96 - DNA, 354 bp, Artificial
  42Y073-86F04-23 variable heavy chain nucleic acid sequence
caggtgcagctggtgcagagcggcgccgaggtgaaaaagcccggcagcagcgtgaaggtgagctgcaaggcctccggcgggaccttcagcggctaccccatcagctgggtgaggcaggctcccggacagggcctggagtggatgggcggcatcatccccattatgggcaccgccaggtacgcccagaagttccagggaagggtcaccatcaccgccgacgagagcaccagcaccgcctacatggaactcagcagcctgaggagcgaggacaccgccgtgtactattgcgccaggctgctgggcgagagcggcatggacgtgtggggccagggcaccaccgtgactgtgagcagc

SEQ ID NO: 97 - protein, 11 aa, Artificial
  CDRL1 amino acid sequence 1
RASQSISSYLN

SEQ ID NO: 98 - protein, 11 aa, Artificial
  CDRL1 amino acid sequence 2
RASQSVSSYLA

SEQ ID NO: 99 - protein, 7 aa, Artificial
  CDRL2 amino acid sequence 1
AASSLQS

SEQ ID NO: 100 - protein, 7 aa, Artificial
  CDRL2 amino acid sequence 2
DASKRAT

SEQ ID NO: 101 - protein, 8 aa, Artificial
  CDRL3 amino acid sequence 1
QQVLHTIT

SEQ ID NO: 102 - protein, 9 aa, Artificial
  CDRL3 amino acid sequence 2
QQPYFSPPT

SEQ ID NO: 103 - protein, 9 aa, Artificial
  CDRL3 amino acid sequence 3
QQLDNWPIT

SEQ ID NO: 104 - protein, 9 aa, Artificial
  CDRL3 amino acid sequence 4
QQSLYPPRT

SEQ ID NO: 105 - protein, 5 aa, Artificial
  CDRH1 amino acid sequence 1
SYAIS

SEQ ID NO: 106 - protein, 5 aa, Artificial
  CDRH1 amino acid sequence 2
YNAIS

SEQ ID NO: 107 - protein, 5 aa, Artificial
  CDRH1 amino acid sequence 3
SEAIS

SEQ ID NO: 108 - protein, 5 aa, Artificial
  CDRH1 amino acid sequence 4
SHAIS

SEQ ID NO: 109 - protein, 5 aa, Artificial
  CDRH1 amino acid sequence 5
GHAIS

SEQ ID NO: 110 - protein, 5 aa, Artificial
  CDRH1 amino acid sequence 6
SRAIS

SEQ ID NO: 111 - protein, 5 aa, Artificial
  CDRH1 amino acid sequence 7
SSAIS

SEQ ID NO: 112 - protein, 5 aa, Artificial
  CDRH1 amino acid sequence 8
NYAIS

SEQ ID NO: 113 - protein, 5 aa, Artificial
  CDRH1 amino acid sequence 9
EYAIH

SEQ ID NO: 114 - protein, 5 aa, Artificial
  CDRH1 amino acid sequence 10
LYAIS

SEQ ID NO: 115 - protein, 5 aa, Artificial
  CDRH1 amino acid sequence 11
EYAIS

SEQ ID NO: 116 - protein, 5 aa, Artificial
  CDRH1 amino acid sequence 12
SYAMH

SEQ ID NO: 117 - protein, 5 aa, Artificial
  CDRH1 amino acid sequence 13
QYAIH

SEQ ID NO: 118 - protein, 5 aa, Artificial
  CDRH1 amino acid sequence 14
RYYWS

SEQ ID NO: 119 - protein, 5 aa, Artificial
  CDRH1 amino acid sequence 15
SYPMH

SEQ ID NO: 120 - protein, 5 aa, Artificial
  CDRH1 amino acid sequence 16
RAAMH

SEQ ID NO: 121 - protein, 5 aa, Artificial
  CDRH1 amino acid sequence 17
TYRMH

SEQ ID NO: 122 - protein, 5 aa, Artificial
  CDRH1 amino acid sequence 18
AYQMH

SEQ ID NO: 123 - protein, 5 aa, Artificial
  CDRH1 amino acid sequence 19
RYNMH

SEQ ID NO: 124 - protein, 5 aa, Artificial
  CDRH1 amino acid sequence 20
KYRMH

SEQ ID NO: 125 - protein, 5 aa, Artificial
  CDRH1 amino acid sequence 21
GYPIS

SEQ ID NO: 126 - protein, 17 aa, Artificial
  CDRH2 amino acid sequence 1
GIIPIFGTASYAQKFQG

SEQ ID NO: 127 - protein, 17 aa, Artificial
  CDRH2 amino acid sequence 2
GIIPIMGTARYAQKFQG

SEQ ID NO: 128 - protein, 17 aa, Artificial
  CDRH2 amino acid sequence 3
GIIPIFGRARYAQKFQG

SEQ ID NO: 129 - protein, 17 aa, Artificial
  CDRH2 amino acid sequence 4
GIIPIFGRGKYAQKFQG

SEQ ID NO: 130 - protein, 17 aa, Artificial
  CDRH2 amino acid sequence 5
GILPIFGRANYAQKFQG

SEQ ID NO: 131 - protein, 17 aa, Artificial
  CDRH2 amino acid sequence 6
GIIPIFGRANYAQKFQG

SEQ ID NO: 132 - protein, 17 aa, Artificial
  CDRH2 amino acid sequence 7
GIIPALGTANYAQKFQG

SEQ ID NO: 133 - protein, 17 aa, Artificial
  CDRH2 amino acid sequence 8
NIIPIFGTAGYAQKFQG

SEQ ID NO: 134 - protein, 17 aa, Artificial
  CDRH2 amino acid sequence 9
GIIPQLGTANYAQKFQG

SEQ ID NO: 135 - protein, 17 aa, Artificial
  CDRH2 amino acid sequence 10
GIIPVFGTANYAQKFQG

SEQ ID NO: 136 - protein, 17 aa, Artificial
  CDRH2 amino acid sequence 11
GIIPIFGTAWYAQKFQG

SEQ ID NO: 137 - protein, 17 aa, Artificial
  CDRH2 amino acid sequence 12
VIIPIFGKANYAQKFQG

SEQ ID NO: 138 - protein, 16 aa, Artificial
  CDRH2 amino acid sequence 13
EIDGWGSTNYNPSLKS

SEQ ID NO: 139 - protein, 17 aa, Artificial
  CDRH2 amino acid sequence 14
IINPSGGFTSYAQKFQG

SEQ ID NO: 140 - protein, 17 aa, Artificial
  CDRH2 amino acid sequence 15
IINPAGGYTSYAQKFQG

SEQ ID NO: 141 - protein, 17 aa, Artificial
  CDRH2 amino acid sequence 16
IINPSGGLTQYAQKFQG

SEQ ID NO: 142 - protein, 17 aa, Artificial
  CDRH2 amino acid sequence 17
IINPAGGWTSYAQKFQG

SEQ ID NO: 143 - protein, 17 aa, Artificial
  CDRH2 amino acid sequence 18
WINPAGGSTSYAQKFQG

SEQ ID NO: 144 - protein, 17 aa, Artificial
  CDRH2 amino acid sequence 19
IINPQGGSTSYAQKFQG

SEQ ID NO: 145 - protein, 17 aa, Artificial
  CDRH2 amino acid sequence 20
GIIPAFGTAQYAQKFQG

SEQ ID NO: 146 - protein, 17 aa, Artificial
  CDRH2 amino acid sequence 21
GIVPVFGTAKYAQKFQG

SEQ ID NO: 147 - protein, 13 aa, Artificial
  CDRH3 amino acid sequence 1
GAGYYGDKDPMDV

SEQ ID NO: 148 - protein, 9 aa, Artificial
  CDRH3 amino acid sequence 2
LLGESGMDV

SEQ ID NO: 149 - protein, 18 aa, Artificial
  CDRH3 amino acid sequence 3
GGSVDFWSGSDYYYYMDV

SEQ ID NO: 150 - protein, 14 aa, Artificial
  CDRH3 amino acid sequence 4
ETAYYTTKGNWFDP

SEQ ID NO: 151 - protein, 5 aa, Artificial
  PD-1 antagonist CDRH1
SYDMS

SEQ ID NO: 152 - protein, 17 aa, Artificial
  PD-1 antagonist CDRH2
TISGGGSYTYYQDSVKG

SEQ ID NO: 153 - protein, 7 aa, Artificial
  PD-1 antagonist CDRH3
PYYAMDY

SEQ ID NO: 154 - protein, 11 aa, Artificial
  PD-1 antagonist CDRL1
KASQDVGTAVA

SEQ ID NO: 155 - protein, 7 aa, Artificial
  PD-1 antagonist CDRL2
WASTLHT

SEQ ID NO: 156 - protein, 9 aa, Artificial
  PD-1 antagonist CDRH3
QHYSSYPWT

SEQ ID NO: 157 - protein, 9 aa, Artificial
  PD-1 antagonist alternative CDRL3
QHYNSYPWT

SEQ ID NO: 158 - protein, 116 aa, Artificial
  PD-1 antagonist heavy chain variable region
EVQLLESGGGLVQPGGSLRLSCAASGFTFSSYDMSWVRQAPGKGLEWVSTISGGGSYTYYQDSVKGRFTISRDNSKNTLYLQMNSLRAEDTAVYYCASPYYAMDYWGQGTTVTVSS

SEQ ID NO: 159 - protein, 107 aa, Artificial
  PD-1 antagonist light chain variable region
DIQLTQSPSFLSAYVGDRVTITCKASQDVGTAVAWYQQKPGKAPKLLIYWASTLHTGVPSRFSGSGSGTEFTLTISSLQPEDFATYYCQHYSSYPWTFGQGTKLEIK

SEQ ID NO: 160 - protein, 443 aa, Artificial
  PD-1 antagonist monoclonal antibody heavy chain
EVQLLESGGGLVQPGGSLRLSCAASGFTFSSYDMSWVRQAPGKGLEWVSTISGGGSYTYYQDSVKGRFTISRDNSKNTLYLQMNSLRAEDTAVYYCASPYYAMDYWGQGTTVTVSSASTKGPSVFPLAPCSRSTSESTAALGCLVKDYFPEPVTVSWNSGALTSGVHTFPAVLQSSGLYSLSSVVTVPSSSLGTKTYTCNVDHKPSNTKVDKRVESKYGPPCPPCPAPEFLGGPSVFLFPPKPKDTLMISRTPEVTCVVVDVSQEDPEVQFNWYVDGVEVHNAKTKPREEQFNSTYRVVSVLTVLHQDWLNGKEYKCKVSNKGLPSSIEKTISKAKGQPREPQVYTLPPSQEEMTKNQVSLTCLVKGFYPSDIAVEWESNGQPENNYKTTPPVLDSDGSFFLYSRLTVDKSRWQEGNVFSCSVMHEALHNHYTQKSLSLSLGK

SEQ ID NO: 161 - protein, 214 aa, Artificial
  PD-1 antagonist monoclonal antibody light chain
DIQLTQSPSFLSAYVGDRVTITCKASQDVGTAVAWYQQKPGKAPKLLIYWASTLHTGVPSRFSGSGSGTEFTLTISSLQPEDFATYYCQHYSSYPWTFGQGTKLEIKRTVAAPSVFIFPPSDEQLKSGTASVVCLLNNFYPREAKVQWKVDNALQSGNSQESVTEQDSKDSTYSLSSTLTLSKADYEKHKVYACEVTHQGLSSPVTKSFNRGEC

SEQ ID NO: 162 - protein, 443 aa, Artificial
  PD-1 antagonist heavy chain sequence with N380D modification
EVQLLESGGGLVQPGGSLRLSCAASGFTFSSYDMSWVRQAPGKGLEWVSTISGGGSYTYYQDSVKGRFTISRDNSKNTLYLQMNSLRAEDTAVYYCASPYYAMDYWGQGTTVTVSSASTKGPSVFPLAPCSRSTSESTAALGCLVKDYFPEPVTVSWNSGALTSGVHTFPAVLQSSGLYSLSSVVTVPSSSLGTKTYTCNVDHKPSNTKVDKRVESKYGPPCPPCPAPEFLGGPSVFLFPPKPKDTLMISRTPEVTCVVVDVSQEDPEVQFNWYVDGVEVHNAKTKPREEQFNSTYRVVSVLTVLHQDWLNGKEYKCKVSNKGLPSSIEKTISKAKGQPREPQVYTLPPSQEEMTKNQVSLTCLVKGFYPSDIAVEWESDGQPENNYKTTPPVLDSDGSFFLYSRLTVDKSRWQEGNVFSCSVMHEALHNHYTQKSLSLSLGK

SEQ ID NO: 163 - protein, 443 aa, Artificial
  PD-1 antagonist light chain sequence with N385D modification
EVQLLESGGGLVQPGGSLRLSCAASGFTFSSYDMSWVRQAPGKGLEWVSTISGGGSYTYYQDSVKGRFTISRDNSKNTLYLQMNSLRAEDTAVYYCASPYYAMDYWGQGTTVTVSSASTKGPSVFPLAPCSRSTSESTAALGCLVKDYFPEPVTVSWNSGALTSGVHTFPAVLQSSGLYSLSSVVTVPSSSLGTKTYTCNVDHKPSNTKVDKRVESKYGPPCPPCPAPEFLGGPSVFLFPPKPKDTLMISRTPEVTCVVVDVSQEDPEVQFNWYVDGVEVHNAKTKPREEQFNSTYRVVSVLTVLHQDWLNGKEYKCKVSNKGLPSSIEKTISKAKGQPREPQVYTLPPSQEEMTKNQVSLTCLVKGFYPSDIAVEWESNGQPEDNYKTTPPVLDSDGSFFLYSRLTVDKSRWQEGNVFSCSVMHEALHNHYTQKSLSLSLGK

SEQ ID NO: 164 - protein, 443 aa, Artificial
  PD-1 antagonist heavy chain sequence with N380D and N385D modifications
EVQLLESGGGLVQPGGSLRLSCAASGFTFSSYDMSWVRQAPGKGLEWVSTISGGGSYTYYQDSVKGRFTISRDNSKNTLYLQMNSLRAEDTAVYYCASPYYAMDYWGQGTTVTVSSASTKGPSVFPLAPCSRSTSESTAALGCLVKDYFPEPVTVSWNSGALTSGVHTFPAVLQSSGLYSLSSVVTVPSSSLGTKTYTCNVDHKPSNTKVDKRVESKYGPPCPPCPAPEFLGGPSVFLFPPKPKDTLMISRTPEVTCVVVDVSQEDPEVQFNWYVDGVEVHNAKTKPREEQFNSTYRVVSVLTVLHQDWLNGKEYKCKVSNKGLPSSIEKTISKAKGQPREPQVYTLPPSQEEMTKNQVSLTCLVKGFYPSDIAVEWESDGQPEDNYKTTPPVLDSDGSFFLYSRLTVDKSRWQEGNVFSCSVMHEALHNHYTQKSLSLSLGK

SEQ ID NO: 165 - protein, 452 aa, Artificial
  42Y073-86F08-66 full length heavy chain amino acid sequence
QVQLVQSGAEVKKPGSSVKVSCKASGGTFVEYAISWVRQAPGQGLEWMGGIIPAFGTAQYAQKFQGRVTITADESTSTAYMELSSLRSEDTAVYYCARGAGYYGDKDPMDVWGQGTTVTVSSASTKGPSVFPLAPSSKSTSGGTAALGCLVKDYFPEPVTVSWNSGALTSGVHTFPAVLQSSGLYSLSSVVTVPSSSLGTQTYICNVNHKPSNTKVDKKVEPKSCDKTHTCPPCPAPELLGGPSVFLFPPKPKDTLMISRTPEVTCVVVDVSHEDPEVKFNWYVDGVEVHNAKTKPREEQYNSTYRVVSVLTVLHQDWLNGKEYKCKVSNKALPAPIEKTISKAKGQPREPQVYTLPPSRDELTKNQVSLTCLVKGFYPSDIAVEWESNGQPENNYKTTPPVLDSDGSFFLYSKLTVDKSRWQQGNVFSCSVMHEALHNHYTQKSLSLSPGK

SEQ ID NO: 166 - protein, 213 aa, Artificial
  42Y073-86F08-66 full length light chain amino acid sequence
DIQLTQSPSSLSASVGDRVTITCRASQSISSYLNWYQQKPGKAPKLLIYAASSLQSGVPSRFSGSGSGTDFTLTISSLQPEDFATYYCQQVLHTITFGGGTKVEIKRTVAAPSVFIFPPSDEQLKSGTASVVCLLNNFYPREAKVQWKVDNALQSGNSQESVTEQDSKDSTYSLSSTLTLSKADYEKHKVYACEVTHQGLSSPVTKSFNRGEC

SEQ ID NO: 167 - DNA, 1356 bp, Artificial
  42Y073-86F08-66 full length heavy chain DNA sequence
caggtgcagctggtgcagagcggcgcagaggtgaaaaagcccggcagcagcgtgaaggtgagctgcaaggcctccggcgggaccttcgtggagtacgccatcagctgggtgaggcaggctcccggacagggcctggagtggatgggcggcatcatccccgccttcggcaccgcccagtacgcccagaagttccagggaagggtcaccatcaccgccgacgagagcaccagcaccgcctacatggaactcagcagcctgaggagcgaggacaccgccgtgtactattgcgccaggggagccggctactacggcgacaaggaccccatggacgtgtggggccagggcaccaccgtgactgtgagcagcgccagcaccaagggccccagcgtgttccccctggcccccagcagcaagagcaccagcggcggcacagccgccctgggctgcctggtgaaggactacttccccgagcccgtgaccgtgtcctggaacagcggagccctgaccagcggcgtgcacaccttccccgccgtgctgcagagcagcggcctgtacagcctgagcagcgtggtgaccgtgcccagcagcagcctgggcacccagacctacatctgtaacgtgaaccacaagcccagcaacaccaaggtggacaagaaggtggagcccaagagctgtgacaagacccacacctgccccccctgccctgcccccgagctgctgggaggccccagcgtgttcctgttcccccccaagcctaaggacaccctgatgatcagcagaacccccgaggtgacctgtgtggtggtggatgtgagccacgaggaccctgaggtgaagttcaactggtacgtggacggcgtggaggtgcacaatgccaagaccaagcccagggaggagcagtacaacagcacctaccgggtggtgtccgtgctgaccgtgctgcaccaggattggctgaacggcaaggagtacaagtgtaaggtgtccaacaaggccctgcctgcccctatcgagaaaaccatcagcaaggccaagggccagcccagagagccccaggtgtacaccctgccccctagcagagatgagctgaccaagaaccaggtgtccctgacctgcctggtgaagggcttctaccccagcgacatcgccgtggagtgggagagcaacggccagcccgagaacaactacaagaccaccccccctgtgctggacagcgatggcagcttcttcctgtacagcaagctgaccgtggacaagagcagatggcagcagggcaacgtgttcagctgctccgtgatgcacgaggccctgcacaatcactacacccagaagagcctgagcctgtcccctggcaag

SEQ ID NO: 168 - DNA, 639 bp, Artificial
  42Y073-86F08-66 full length light chain DNA sequence
gacatccagctgacccagagccctagcagcctgagcgccagcgtgggagacagggtgaccatcacctgcagggccagccagtccatcagcagctacctgaactggtaccagcagaagcccggcaaggcccccaagctgctgatctacgccgcaagctcactgcagagcggcgtgccctctaggtttagcggcagcggcagcggcaccgacttcaccctgaccatcagcagcctccagcccgaggacttcgccacctactactgccagcaggtgctgcacaccatcactttcggcggcggcaccaaggtggagattaagcgtacggtggccgcccccagcgtgttcatcttcccccccagcgatgagcagctgaagagcggcaccgccagcgtggtgtgtctgctgaacaacttctacccccgggaggccaaggtgcagtggaaggtggacaatgccctgcagagcggcaacagccaggagagcgtgaccgagcaggacagcaaggactccacctacagcctgagcagcaccctgaccctgagcaaggccgactacgagaagcacaaggtgtacgcctgtgaggtgacccaccagggcctgtccagccccgtgaccaagagcttcaaccggggcgagtgc

SEQ ID NO: 169 - protein, 213 aa, Artificial; identical to SEQ ID NO: 166
  42Y073-86F08-16 full length light chain amino acid sequence

SEQ ID NO: 170 - protein, 452 aa, Artificial
  42Y073-86F08-16 full length heavy chain amino acid sequence
QVQLVQSGAEVKKPGSSVKVSCKASGGTFNEYAISWVRQAPGQGLEWMGGIVPVFGTAKYAQKFQGRVTITADESTSTAYMELSSLRSEDTAVYYCARGAGYYGDKDPMDVWGQGTTVTVSSASTKGPSVFPLAPSSKSTSGGTAALGCLVKDYFPEPVTVSWNSGALTSGVHTFPAVLQSSGLYSLSSVVTVPSSSLGTQTYICNVNHKPSNTKVDKKVEPKSCDKTHTCPPCPAPELLGGPSVFLFPPKPKDTLMISRTPEVTCVVVDVSHEDPEVKFNWYVDGVEVHNAKTKPREEQYNSTYRVVSVLTVLHQDWLNGKEYKCKVSNKALPAPIEKTISKAKGQPREPQVYTLPPSRDELTKNQVSLTCLVKGFYPSDIAVEWESNGQPENNYKTTPPVLDSDGSFFLYSKLTVDKSRWQQGNVFSCSVMHEALHNHYTQKSLSLSPGK

SEQ ID NO: 171 - DNA, 639 bp, Artificial; identical to SEQ ID NO: 168
  42Y073-86F08-16 full length light chain DNA sequence

SEQ ID NO: 172 - DNA, 1356 bp, Artificial
  42Y073-86F08-16  full length heavy chain DNA sequence
caggtgcagctggtgcagagcggcgccgaggtgaaaaagcccggcagcagcgtgaaggtgagctgcaaggcctccggcgggaccttcaacgagtacgccatcagctgggtgaggcaggctcccggacagggcctggagtggatgggcggcatcgtgcccgtgttcggcaccgccaagtacgcccagaagttccagggaagggtcaccatcaccgccgacgagagcaccagcaccgcctacatggaactcagcagcctgaggagcgaggacaccgccgtgtactattgcgccaggggcgccggctactacggcgacaaggaccccatggacgtgtggggccagggcaccaccgtgactgtgagcagcgccagcaccaagggccccagcgtgttccccctggcccccagcagcaagagcaccagcggcggcacagccgccctgggctgcctggtgaaggactacttccccgagcccgtgaccgtgtcctggaacagcggagccctgaccagcggcgtgcacaccttccccgccgtgctgcagagcagcggcctgtacagcctgagcagcgtggtgaccgtgcccagcagcagcctgggcacccagacctacatctgtaacgtgaaccacaagcccagcaacaccaaggtggacaagaaggtggagcccaagagctgtgacaagacccacacctgccccccctgccctgcccccgagctgctgggaggccccagcgtgttcctgttcccccccaagcctaaggacaccctgatgatcagcagaacccccgaggtgacctgtgtggtggtggatgtgagccacgaggaccctgaggtgaagttcaactggtacgtggacggcgtggaggtgcacaatgccaagaccaagcccagggaggagcagtacaacagcacctaccgggtggtgtccgtgctgaccgtgctgcaccaggattggctgaacggcaaggagtacaagtgtaaggtgtccaacaaggccctgcctgcccctatcgagaaaaccatcagcaaggccaagggccagcccagagagccccaggtgtacaccctgccccctagcagagatgagctgaccaagaaccaggtgtccctgacctgcctggtgaagggcttctaccccagcgacatcgccgtggagtgggagagcaacggccagcccgagaacaactacaagaccaccccccctgtgctggacagcgatggcagcttcttcctgtacagcaagctgaccgtggacaagagcagatggcagcagggcaacgtgttcagctgctccgtgatgcacgaggccctgcacaatcactacacccagaagagcctgagcctgtcccctggcaag

SEQ ID NO: 173 - protein, 214 aa, Artificial
  42Y073-86F04-23 full length light chain amino acid sequence
DIQMTQSPSSLSASVGDRVTITCRASQSISSYLNWYQQKPGKAPKLLIYAASSLQSGVPSRFSGSGSGTDFTLTISSLQPEDFATYYCQQPYFSPPTFGGGTKVEIKRTVAAPSVFIFPPSDEQLKSGTASVVCLLNNFYPREAKVQWKVDNALQSGNSQESVTEQDSKDSTYSLSSTLTLSKADYEKHKVYACEVTHQGLSSPVTKSFNRGEC

SEQ ID NO: 174 - protein, 448 aa, Artificial
  42Y073-86F04-23 full length Heavy chain amino acid sequence
QVQLVQSGAEVKKPGSSVKVSCKASGGTFSGYPISWVRQAPGQGLEWMGGIIPIMGTARYAQKFQGRVTITADESTSTAYMELSSLRSEDTAVYYCARLLGESGMDVWGQGTTVTVSSASTKGPSVFPLAPSSKSTSGGTAALGCLVKDYFPEPVTVSWNSGALTSGVHTFPAVLQSSGLYSLSSVVTVPSSSLGTQTYICNVNHKPSNTKVDKKVEPKSCDKTHTCPPCPAPELLGGPSVFLFPPKPKDTLMISRTPEVTCVVVDVSHEDPEVKFNWYVDGVEVHNAKTKPREEQYNSTYRVVSVLTVLHQDWLNGKEYKCKVSNKALPAPIEKTISKAKGQPREPQVYTLPPSRDELTKNQVSLTCLVKGFYPSDIAVEWESNGQPENNYKTTPPVLDSDGSFFLYSKLTVDKSRWQQGNVFSCSVMHEALHNHYTQKSLSLSPGK

SEQ ID NO: 175 - DNA, 642 bp, Artificial
  42Y073-86F04-23 full length Light chain DNA sequence
gacatccagatgacccagagccctagcagcctgagcgccagcgtgggagacagggtgaccatcacctgcagggccagccagtccatcagcagctacctgaactggtaccagcagaagcccggcaaggcccccaagctgctgatctacgccgcaagctcactgcagagcggcgtgccctctaggtttagcggcagcggcagcggcaccgacttcaccctgaccatcagcagcctccagcccgaggacttcgccacctactactgccagcagccctacttcagcccccccactttcggcggcggcaccaaggtggagattaagcgtacggtggccgcccccagcgtgttcatcttcccccccagcgatgagcagctgaagagcggcaccgccagcgtggtgtgtctgctgaacaacttctacccccgggaggccaaggtgcagtggaaggtggacaatgccctgcagagcggcaacagccaggagagcgtgaccgagcaggacagcaaggactccacctacagcctgagcagcaccctgaccctgagcaaggccgactacgagaagcacaaggtgtacgcctgtgaggtgacccaccagggcctgtccagccccgtgaccaagagcttcaaccggggcgagtgc

SEQ ID NO: 176 - DNA, 1344 bp, Artificial
  42Y073-86F04-23  full length Heavy chain DNA sequence
caggtgcagctggtgcagagcggcgccgaggtgaaaaagcccggcagcagcgtgaaggtgagctgcaaggcctccggcgggaccttcagcggctaccccatcagctgggtgaggcaggctcccggacagggcctggagtggatgggcggcatcatccccattatgggcaccgccaggtacgcccagaagttccagggaagggtcaccatcaccgccgacgagagcaccagcaccgcctacatggaactcagcagcctgaggagcgaggacaccgccgtgtactattgcgccaggctgctgggcgagagcggcatggacgtgtggggccagggcaccaccgtgactgtgagcagcgccagcaccaagggccccagcgtgttccccctggcccccagcagcaagagcaccagcggcggcacagccgccctgggctgcctggtgaaggactacttccccgagcccgtgaccgtgtcctggaacagcggagccctgaccagcggcgtgcacaccttccccgccgtgctgcagagcagcggcctgtacagcctgagcagcgtggtgaccgtgcccagcagcagcctgggcacccagacctacatctgtaacgtgaaccacaagcccagcaacaccaaggtggacaagaaggtggagcccaagagctgtgacaagacccacacctgccccccctgccctgcccccgagctgctgggaggccccagcgtgttcctgttcccccccaagcctaaggacaccctgatgatcagcagaacccccgaggtgacctgtgtggtggtggatgtgagccacgaggaccctgaggtgaagttcaactggtacgtggacggcgtggaggtgcacaatgccaagaccaagcccagggaggagcagtacaacagcacctaccgggtggtgtccgtgctgaccgtgctgcaccaggattggctgaacggcaaggagtacaagtgtaaggtgtccaacaaggccctgcctgcccctatcgagaaaaccatcagcaaggccaagggccagcccagagagccccaggtgtacaccctgccccctagcagagatgagctgaccaagaaccaggtgtccctgacctgcctggtgaagggcttctaccccagcgacatcgccgtggagtgggagagcaacggccagcccgagaacaactacaagaccaccccccctgtgctggacagcgatggcagcttcttcctgtacagcaagctgaccgtggacaagagcagatggcagcagggcaacgtgttcagctgctccgtgatgcacgaggccctgcacaatcactacacccagaagagcctgagcctgtcccctggcaag

SEQ ID NO: 177 - protein, 564 aa, Artificial Sequence
  CD155-fc amino acid sequence used in examples
WPPPGTGDVVVQAPTQVPGFLGDSVTLPCYLQVPNMEVTHVSQLTWARHGESGSMAVFHQTQGPSYSESKRLEFVAARLGAELRNASLRMFGLRVEDEGNYTCLFVTFPQGSRSVDIWLRVLAKPQNTAEVQKVQLTGEPVPMARCVSTGGRPPAQITWHSDLGGMPNTSQVPGFLSGTVTVTSLWILVPSSQVDGKNVTCKVEHESFEKPQLLTVNLTVYYPPEVSISGYDNNWYLGQNEATLTCDARSNPEPTGYNWSTTMGPLPPFAVAQGAQLLIRPVDKPINTTLICNVTNALGARQAELTVQVKEGPPSEHSGISRNSGENLYFQGDPKSCDKTHTCPPCPAPELLGGPSVFLFPPKPKDTLMISRTPEVTCVVVDVSHEDPEVKFNWYVDGVEVHNAKTKPREEQYNSTYRVVSVLTVLHQDWLNGKEYKCKVSNKALPAPIEKTISKAKGQPREPQVYTLPPSRDELTKNQVSLTCLVKGFYPSDIAVEWESNGQPENNYKTTPPVLDSDGSFFLYSKLTVDKSRWQQGNVFSCSVMHEALHNHYTQKSLSLSPGK

SEQ ID NO: 178 - protein, 417 aa, Homo sapiens
MARAMAAAWPLLLVALLVLSWPPPGTGDVVVQAPTQVPGFLGDSVTLPCYLQVPNMEVTHVSQLTWARHGESGSMAVFHQTQGPSYSESKRLEFVAARLGAELRNASLRMFGLRVEDEGNYTCLFVTFPQGSRSVDIWLRVLAKPQNTAEVQKVQLTGEPVPMARCVSTGGRPPAQITWHSDLGGMPNTSQVPGFLSGTVTVTSLWILVPSSQVDGKNVTCKVEHESFEKPQLLTVNLTVYYPPEVSISGYDNNWYLGQNEATLTCDARSNPEPTGYNWSTTMGPLPPFAVAQGAQLLIRPVDKPINTTLICNVTNALGARQAELTVQVKEGPPSEHSGISRNAIIFLVLGILVFLILLGIGIYFYWSKCSREVLWHCHLCPSSTEHASASANGHVSYSAVSRENSSSQDPQTEGTR

SEQ ID NO: 179 - protein, 330 aa, Homo sapiens [sequence omitted]

SEQ ID NO: 180 - DNA, 990 bp, Homo sapiens
gccagcaccaagggccccagcgtgttccccctggcccccagcagcaagagcaccagcggcggcacagccgccctgggctgcctggtgaaggactacttccccgagcccgtgaccgtgtcctggaacagcggagccctgaccagcggcgtgcacaccttccccgccgtgctgcagagcagcggcctgtacagcctgagcagcgtggtgaccgtgcccagcagcagcctgggcacccagacctacatctgtaacgtgaaccacaagcccagcaacaccaaggtggacaagaaggtggagcccaagagctgtgacaagacccacacctgccccccctgccctgcccccgagctgctgggaggccccagcgtgttcctgttcccccccaagcctaaggacaccctgatgatcagcagaacccccgaggtgacctgtgtggtggtggatgtgagccacgaggaccctgaggtgaagttcaactggtacgtggacggcgtggaggtgcacaatgccaagaccaagcccagggaggagcagtacaacagcacctaccgggtggtgtccgtgctgaccgtgctgcaccaggattggctgaacggcaaggagtacaagtgtaaggtgtccaacaaggccctgcctgcccctatcgagaaaaccatcagcaaggccaagggccagcccagagagccccaggtgtacaccctgccccctagcagagatgagctgaccaagaaccaggtgtccctgacctgcctggtgaagggcttctaccccagcgacatcgccgtggagtgggagagcaacggccagcccgagaacaactacaagaccaccccccctgtgctggacagcgatggcagcttcttcctgtacagcaagctgaccgtggacaagagcagatggcagcagggcaacgtgttcagctgctccgtgatgcacgaggccctgcacaatcactacacccagaagagcctgagcctgtcccctggcaag